European Patent Application EP 4 273 168 A1, published November 8, 2023. Title: ANTIBODY THAT SPECIFICALLY BINDS TO BCMA AND USE THEREOF. Applicant: IMMUNOCHINA PHARMACEUTICALS CO., LTD BEIJING YIMIAOYILIAO CO., LTD. The sequence listing filed with the application follows.

SEQUENCE LISTING (56 sequences)

SEQ ID NO: 1 - protein, 10 aa, Artificial Sequence
  UNSURE (5)..(5): Ser or Thr or Arg
  UNSURE (6)..(6): Arg or Ser or His
  PEPTIDE (1)..(10): VH-CDR1
GYTFXXYSMN

SEQ ID NO: 3 - protein, 17 aa, Artificial Sequence
  UNSURE (5)..(5): Gly or Glu or Arg
  UNSURE (8)..(8): Ala or Thr or Val
  UNSURE (10)..(10): Ile or Asn
  PEPTIDE (1)..(17): VH-CDR2
RINTXSGXPXYADDFKG

SEQ ID NO: 3 - protein, 10 aa, Artificial Sequence
  UNSURE (5)..(5): Asn or Leu
  UNSURE (10)..(10): His or Tyr or Phe
  PEPTIDE (1)..(10): VH-CDR3
SNDYXYSLDX

SEQ ID NO: 4 - protein, 15 aa, Artificial Sequence
  UNSURE (4)..(4): Arg or Glu
  UNSURE (7)..(7): Thr or Ser
  UNSURE (8)..(8): Ile or Val
  UNSURE (9)..(9): Ala or Leu
  UNSURE (11)..(11): Ser or Asn
  UNSURE (12)..(12): Pro or His
  UNSURE (13)..(13): Ile or Leu
  UNSURE (14)..(14): Ile or Val
  PEPTIDE (1)..(15): VL-CDR1
RASXSVXXXGXXXXY

SEQ ID NO: 5 - protein, 7 aa, Artificial Sequence
  PEPTIDE (1)..(7): VL-CDR2
LASNVQT

SEQ ID NO: 6 - protein, 9 aa, Artificial Sequence
  UNSURE (1)..(1): Leu or Phe
  UNSURE (5)..(5): Thr or Ser
  PEPTIDE (1)..(9): VL-CDR3
XQSRXIPRT

SEQ ID NO: 7 - protein, 10 aa, Artificial Sequence
  PEPTIDE (1)..(10): VH-CDR1
GYTFSRYSMN

SEQ ID NO: 8 - protein, 10 aa, Artificial Sequence
  PEPTIDE (1)..(10): VH-CDR1
GYTFTSYSMN

SEQ ID NO: 9 - protein, 10 aa, Artificial Sequence
  PEPTIDE (1)..(10): VH-CDR1
GYTFRHYSMN

SEQ ID NO: 10 - protein, 17 aa, Artificial Sequence
  PEPTIDE (1)..(17): VH-CDR2
RINTGSGAPIYADDFKG

SEQ ID NO: 11 - protein, 17 aa, Artificial Sequence
  PEPTIDE (1)..(17): VH-CDR2
RINTESGAPNYADDFKG

SEQ ID NO: 12 - protein, 17 aa, Artificial Sequence
  PEPTIDE (1)..(17): VH-CDR2
RINTRSGTPNYADDFKG

SEQ ID NO: 13 - protein, 17 aa, Artificial Sequence
  PEPTIDE (1)..(17): VH-CDR2
RINTESGVPIYADDFKG

SEQ ID NO: 14 - protein, 10 aa, Artificial Sequence
  PEPTIDE (1)..(10): VH-CDR3
SNDYNYSLDH

SEQ ID NO: 15 - protein, 10 aa, Artificial Sequence
  PEPTIDE (1)..(10): VH-CDR3
SNDYLYSLDY

SEQ ID NO: 16 - protein, 10 aa, Artificial Sequence
  PEPTIDE (1)..(10): VH-CDR3
SNDYLYSLDF

SEQ ID NO: 17 - protein, 15 aa, Artificial Sequence
  PEPTIDE (1)..(15): VL-CDR1
RASRSVTILGNPIVY

SEQ ID NO: 18 - protein, 15 aa, Artificial Sequence
  PEPTIDE (1)..(15): VL-CDR1
RASRSVSVAGNHIVY

SEQ ID NO: 19 - protein, 15 aa, Artificial Sequence
  PEPTIDE (1)..(15): VL-CDR1
RASESVTILGSHLIY

SEQ ID NO: 20 - protein, 7 aa, Artificial Sequence
  PEPTIDE (1)..(7): VL-CDR2
LASNVQT

SEQ ID NO: 21 - protein, 9 aa, Artificial Sequence
  PEPTIDE (1)..(9): VL-CDR3
LQSRTIPRT

SEQ ID NO: 22 - protein, 9 aa, Artificial Sequence
  PEPTIDE (1)..(9): VL-CDR3
FQSRSIPRT

SEQ ID NO: 23 - protein, 117 aa, Artificial Sequence
  PEPTIDE (1)..(117): VH
QVQLVQSGPELKKPGETVKISCKASGYTFSRYSMNWVRQAPGKGLEWMGRINTGSGAPIYADDFKGRFIFSVDTSASTAYLVINNLKSEDTASYFCSNDYNYSLDHWGQGTAVTVSS

SEQ ID NO: 24 - protein, 117 aa, Artificial Sequence
  PEPTIDE (1)..(117): VH
QVQLVQSGPELKKPGETVKISCKASGYTFSRYSMNWVRQAPGKGLEWMGRINTGSGAPIYADDFKGRFTFSVDTSASTAYLVINNLKSEDTASYFCSNDYNYSLDHWGQGTAVTVSS

SEQ ID NO: 25 - protein, 117 aa, Artificial Sequence
  PEPTIDE (1)..(117): VH
QVQLVQSGPEVKKPGESVKVSCKASGYTFSRYSMNWVRQAPGQGLEWMGRINTGSGAPIYADDFKGRFTFTVDESTSTAYLVLNNLRSEDTAVYFCSNDYNYSLDHWGQGTAVTVSS

SEQ ID NO: 26 - protein, 117 aa, Artificial Sequence
  PEPTIDE (1)..(117): VH
QVQLVQSGPEVKKPGESVKVSCKASGYTFRHYSMNWVRQAPGQGLEWMGRINTESGVPIYADDFKGRFAFTVDESTSTAYLVLNNLRSEDTAVYFCSNDYLYSLDFWGQGTAVTVSS

SEQ ID NO: 27 - protein, 117 aa, Artificial Sequence
  PEPTIDE (1)..(117): VH
QVQLVQSGPEVKKPGESVKVSCKASGYTFTSYSMNWVRQVPGQGLEWMGRINTESGAPNYADDFKGRFTFTVDTSTSTAYLEINNLRSEDTAVYFCSNDYLYSLDYWGQGTAVTVSS

SEQ ID NO: 28 - protein, 117 aa, Artificial Sequence
  PEPTIDE (1)..(117): VH
QVQLVQSGPELKKPGETVKISCKASGYTFSRYSMNWVRQAPGKGLEWMGRINTGSGAPIYADDFKGRFIFSVDTSASTAYMELSSLRSEDTAVYYCSNDYNYSLDHWGQGTAVTVSS

SEQ ID NO: 29 - protein, 117 aa, Artificial Sequence
  PEPTIDE (1)..(117): VH
QVQLVQSGAEVKKPGASVKVSCKASGYTFTSYSMNWVRQAPGQGLEWMGRINTRSGTPNYADDFKGRVTITADESVSTAYMELSNLKSEDTASYFCSNDYNYSLDHWGQGTAVTVSS

SEQ ID NO: 30 - protein, 117 aa, Artificial Sequence
  PEPTIDE (1)..(117): VH
QVQLVQSGPEVKKPGASVKVSCKASGYTFSRYSMNWVRQAPGQGLEWMGRINTGSGAPIYADDFKGRVTMTRDESTSTAYLVLNNLRSEDTAVYFCSNDYNYSLDHWGQGTAVTVSS

SEQ ID NO: 31 - protein, 117 aa, Artificial Sequence
  PEPTIDE (1)..(117): VH
EVQLVESGGGLVQPGESVKVSCKASGYTFRHYSMNWVRQAPGQGLEWMGRINTESGVPIYADDFKGRFTISRDESTSTAYLVLNNLRSEDTAVYFCSNDYLYSLDFWGQGTAVTVSS

SEQ ID NO: 32 - protein, 117 aa, Artificial Sequence
  PEPTIDE (1)..(117): VH
EVQLVESGGGVKKPGESVKVSCKASGYTFTSYSMNWVRQVPGQGLEWMGRINTESGAPNYADDFKGRFTISRDTSTNSLYLEINNLRSEDTAVYFCSNDYLYSLDYWGQGTAVTVSS

SEQ ID NO: 33 - protein, 111 aa, Artificial Sequence
  PEPTIDE (1)..(111): VL
DIVLTQSPSSLSVSLGQRATISCRASRSVTILGNPIVYWYQQKPGQPPVLLIQLASNVQTGVPARFSGSGSGTDFTLTIDPVEEDDVAVYYCLQSRTIPRTFGGGTKLEIK

SEQ ID NO: 34 - protein, 111 aa, Artificial Sequence
  PEPTIDE (1)..(111): VL
DIVLTQSPSSLSVSLGQRATISCRASRSVTILGNPIVYWYQQKPGQPPVLLIQLASNVQTGVPARFSGSGSGTDFTLTIDPVEEDDVAVYYCFQSRSIPRTFGGGTKLEIK

SEQ ID NO: 35 - protein, 111 aa, Artificial Sequence
  PEPTIDE (1)..(111): VL
EIVLTQSPSTLSVSLGQRATLSCRASRSVTILGNPIVYWYQQKPGQPPVLLIQLASNVQTGIPARFSGSGSGTDFTLTIDPLEEEDVAVYYCLQSRTIPRTFGGGTKLEIK

SEQ ID NO: 36 - protein, 111 aa, Artificial Sequence
  PEPTIDE (1)..(111): VL
EIVLTQSPPTLAMSLGKRATLSCRASESVTILGSHLIYWYQQKPGQPPTLLIQLASNVQTGIPARFSGSGSRTDFTLTIDPLEEEDVAVYYCLQSRTIPRTFGGGTKLEIK

SEQ ID NO: 37 - protein, 111 aa, Artificial Sequence
  PEPTIDE (1)..(111): VL
EIVLTQSPSTLSVSLGQRATLSCRASRSVSVAGNHIVYWYQQKPGQPPVLLIQLASNVQTGIPARFSGSGSGTDFTLTIDSLEPEDVAVYYCLQSRTIPRTFGGGTKLEIK

SEQ ID NO: 38 - protein, 111 aa, Artificial Sequence
  PEPTIDE (1)..(111): VL
EIVLTQSPATLSVSLGQRATISCRASRSVTILGNPIVYWYQQKPGQPPVLLIQLASNVQTGVPARFSGSGSGTDFTLTISSLEEDDVAVYYCLQSRTIPRTFGGGTKLEIK

SEQ ID NO: 39 - protein, 111 aa, Artificial Sequence
  PEPTIDE (1)..(111): VL
EIVMTQSPPTLSVSLGQRATLSCRASRSVTILGNPIVYWYQQKAPKPPVLLIQLASNVQTGIPARFSGSGSGTDFTLTIDPLEEEDVAVYYCLQSRTIPRTFGGGTKLEIK

SEQ ID NO: 40 - protein, 111 aa, Artificial Sequence
  PEPTIDE (1)..(111): 111
EIVLTQSPPTLAMSLGKRATLSCRASESVTILGSHLIYWYQQKPGQPPTLLIQLASNVQTGIPARFSGSGSRTDFTLTIDPLEEEDVAVYYCLQSRTIPRTFGGGTKVEIK

SEQ ID NO: 41 - protein, 111 aa, Artificial Sequence
  PEPTIDE (1)..(111)
EIVLTQSPSTLSVSLGQRATLSCRASRSVSVAGNHIVYWYQQKPGQPPVLLIQLASNVQTGIPARFSGSGSGTDFTLTISSLEPEDVAVYYCLQSRTIPRTFGGGTKLEIK

SEQ ID NO: 42 - protein, 111 aa, Artificial Sequence
  PEPTIDE (1)..(111): VL
EIVLTQSPATLSVSLGQRATISCRASRSVTILGNPIVYWYQQKPGQPPVLLIQLASNVQTGVPARFSGSGSGTDFTLTISSLQSEDFAVYYCLQSRTIPRTFGGGTKLEIK

SEQ ID NO: 43 - protein, 111 aa, Artificial Sequence
  PEPTIDE (1)..(111): VL
DIVLTQSPSSLSVSLGQRATISCRASRSVTILGNPIVYWYQQKPGQPPVLLIQLASNVQTGVPARFSGSGSGTDFTLTISSLQSEDFAVYYCLQSRTIPRTFGGGTKLEIK

SEQ ID NO: 44 - protein, 246 aa, Artificial Sequence
  PEPTIDE (1)..(246): scFv
QVQLVQSGPELKKPGETVKISCKASGYTFSRYSMNWVRQAPGKGLEWMGRINTGSGAPIYADDFKGRFIFSVDTSASTAYLVINNLKSEDTASYFCSNDYNYSLDHWGQGTAVTVSSGSTSGSGKPGSGEGSTKGDIVLTQSPSSLSVSLGQRATISCRASRSVTILGNPIVYWYQQKPGQPPVLLIQLASNVQTGVPARFSGSGSGTDFTLTIDPVEEDDVAVYYCLQSRTIPRTFGGGTKLEIK

SEQ ID NO: 45 - protein, 246 aa, Artificial Sequence
  PEPTIDE (1)..(246): scFv
QVQLVQSGPELKKPGETVKISCKASGYTFSRYSMNWVRQAPGKGLEWMGRINTGSGAPIYADDFKGRFTFSVDTSASTAYLVINNLKSEDTASYFCSNDYNYSLDHWGQGTAVTVSSGSTSGSGKPGSGEGSTKGDIVLTQSPSSLSVSLGQRATISCRASRSVTILGNPIVYWYQQKPGQPPVLLIQLASNVQTGVPARFSGSGSGTDFTLTIDPVEEDDVAVYYCLQSRTIPRTFGGGTKLEIK

SEQ ID NO: 46 - protein, 246 aa, Artificial Sequence
  PEPTIDE (1)..(246): scFv
QVQLVQSGPELKKPGETVKISCKASGYTFSRYSMNWVRQAPGKGLEWMGRINTGSGAPIYADDFKGRFTFSVDTSASTAYLVINNLKSEDTASYFCSNDYNYSLDHWGQGTAVTVSSGSTSGSGKPGSGEGSTKGDIVLTQSPSSLSVSLGQRATISCRASRSVTILGNPIVYWYQQKPGQPPVLLIQLASNVQTGVPARFSGSGSGTDFTLTIDPVEEDDVAVYYCFQSRSIPRTFGGGTKLEIK

SEQ ID NO: 47 - protein, 246 aa, Artificial Sequence
  PEPTIDE (1)..(246): scFv
QVQLVQSGPEVKKPGESVKVSCKASGYTFSRYSMNWVRQAPGQGLEWMGRINTGSGAPIYADDFKGRFTFTVDESTSTAYLVLNNLRSEDTAVYFCSNDYNYSLDHWGQGTAVTVSSGSTSGSGKPGSGEGSTKGEIVLTQSPSTLSVSLGQRATLSCRASRSVTILGNPIVYWYQQKPGQPPVLLIQLASNVQTGIPARFSGSGSGTDFTLTIDPLEEEDVAVYYCLQSRTIPRTFGGGTKLEIK

SEQ ID NO: 48 - protein, 246 aa, Artificial Sequence
  PEPTIDE (1)..(246): scFv
QVQLVQSGPEVKKPGESVKVSCKASGYTFRHYSMNWVRQAPGQGLEWMGRINTESGVPIYADDFKGRFAFTVDESTSTAYLVLNNLRSEDTAVYFCSNDYLYSLDFWGQGTAVTVSSGSTSGSGKPGSGEGSTKGEIVLTQSPPTLAMSLGKRATLSCRASESVTILGSHLIYWYQQKPGQPPTLLIQLASNVQTGIPARFSGSGSRTDFTLTIDPLEEEDVAVYYCLQSRTIPRTFGGGTKLEIK

SEQ ID NO: 49 - protein, 246 aa, Artificial Sequence
  PEPTIDE (1)..(246): scFv
QVQLVQSGPEVKKPGESVKVSCKASGYTFTSYSMNWVRQVPGQGLEWMGRINTESGAPNYADDFKGRFTFTVDTSTSTAYLEINNLRSEDTAVYFCSNDYLYSLDYWGQGTAVTVSSGSTSGSGKPGSGEGSTKGEIVLTQSPSTLSVSLGQRATLSCRASRSVSVAGNHIVYWYQQKPGQPPVLLIQLASNVQTGIPARFSGSGSGTDFTLTIDSLEPEDVAVYYCLQSRTIPRTFGGGTKLEIK

SEQ ID NO: 50 - protein, 246 aa, Artificial Sequence
  PEPTIDE (1)..(246): scFv
QVQLVQSGPELKKPGETVKISCKASGYTFSRYSMNWVRQAPGKGLEWMGRINTGSGAPIYADDFKGRFIFSVDTSASTAYMELSSLRSEDTAVYYCSNDYNYSLDHWGQGTAVTVSSGSTSGSGKPGSGEGSTKGEIVLTQSPATLSVSLGQRATISCRASRSVTILGNPIVYWYQQKPGQPPVLLIQLASNVQTGVPARFSGSGSGTDFTLTISSLEEDDVAVYYCLQSRTIPRTFGGGTKLEIK

SEQ ID NO: 51 - protein, 246 aa, Artificial Sequence
  PEPTIDE (1)..(246): scFv
QVQLVQSGAEVKKPGASVKVSCKASGYTFTSYSMNWVRQAPGQGLEWMGRINTRSGTPNYADDFKGRVTITADESVSTAYMELSNLKSEDTASYFCSNDYNYSLDHWGQGTAVTVSSGSTSGSGKPGSGEGSTKGDIVLTQSPSSLSVSLGQRATISCRASRSVTILGNPIVYWYQQKPGQPPVLLIQLASNVQTGVPARFSGSGSGTDFTLTIDPVEEDDVAVYYCLQSRTIPRTFGGGTKLEIK

SEQ ID NO: 52 - protein, 246 aa, Artificial Sequence
  PEPTIDE (1)..(246): scFv
QVQLVQSGPEVKKPGASVKVSCKASGYTFSRYSMNWVRQAPGQGLEWMGRINTGSGAPIYADDFKGRVTMTRDESTSTAYLVLNNLRSEDTAVYFCSNDYNYSLDHWGQGTAVTVSSGSTSGSGKPGSGEGSTKGEIVMTQSPPTLSVSLGQRATLSCRASRSVTILGNPIVYWYQQKAPKPPVLLIQLASNVQTGIPARFSGSGSGTDFTLTIDPLEEEDVAVYYCLQSRTIPRTFGGGTKLEIK

SEQ ID NO: 53 - protein, 246 aa, Artificial Sequence
  PEPTIDE (1)..(246): scFv
EVQLVESGGGLVQPGESVKVSCKASGYTFRHYSMNWVRQAPGQGLEWMGRINTESGVPIYADDFKGRFTISRDESTSTAYLVLNNLRSEDTAVYFCSNDYLYSLDFWGQGTAVTVSSGSTSGSGKPGSGEGSTKGEIVLTQSPPTLAMSLGKRATLSCRASESVTILGSHLIYWYQQKPGQPPTLLIQLASNVQTGIPARFSGSGSRTDFTLTIDPLEEEDVAVYYCLQSRTIPRTFGGGTKVEIK

SEQ ID NO: 54 - protein, 246 aa, Artificial Sequence
  PEPTIDE (1)..(246): scFv
EVQLVESGGGVKKPGESVKVSCKASGYTFTSYSMNWVRQVPGQGLEWMGRINTESGAPNYADDFKGRFTISRDTSTNSLYLEINNLRSEDTAVYFCSNDYLYSLDYWGQGTAVTVSSGSTSGSGKPGSGEGSTKGEIVLTQSPSTLSVSLGQRATLSCRASRSVSVAGNHIVYWYQQKPGQPPVLLIQLASNVQTGIPARFSGSGSGTDFTLTISSLEPEDVAVYYCLQSRTIPRTFGGGTKLEIK

SEQ ID NO: 55 - protein, 246 aa, Artificial Sequence
  PEPTIDE (1)..(246): scFv
QVQLVQSGPELKKPGETVKISCKASGYTFSRYSMNWVRQAPGKGLEWMGRINTGSGAPIYADDFKGRFIFSVDTSASTAYMELSSLRSEDTAVYYCSNDYNYSLDHWGQGTAVTVSSGSTSGSGKPGSGEGSTKGEIVLTQSPATLSVSLGQRATISCRASRSVTILGNPIVYWYQQKPGQPPVLLIQLASNVQTGVPARFSGSGSGTDFTLTISSLQSEDFAVYYCLQSRTIPRTFGGGTKLEIK

SEQ ID NO: 56 - protein, 246 aa, Artificial Sequence
  PEPTIDE (1)..(246): scFv
QVQLVQSGAEVKKPGASVKVSCKASGYTFTSYSMNWVRQAPGQGLEWMGRINTRSGTPNYADDFKGRVTITADESVSTAYMELSNLKSEDTASYFCSNDYNYSLDHWGQGTAVTVSSGSTSGSGKPGSGEGSTKGDIVLTQSPSSLSVSLGQRATISCRASRSVTILGNPIVYWYQQKPGQPPVLLIQLASNVQTGVPARFSGSGSGTDFTLTISSLQSEDFAVYYCLQSRTIPRTFGGGTKLEIK